European Patent Application EP 4 253 424 A1, published October 4, 2023. Title: BISPECIFIC ANTIBODY AND USE THEREOF. Applicant: SHANGHAI HUAOTA BIOPHARMACEUTICALCO., LTD.;HUABO BIOPHARM (SHANGHAI) CO., LTD. The sequence listing filed with the application follows.

SEQUENCE LISTING (111 sequences)

SEQ ID NO: 1 - protein, 121 aa, Artificial Sequence
  900424 VH
DVQLQESGPGLVKPSQSLSLTCTVTGYSITSDYAWIWIRQFPGNKVEWMGYITSSGSTSYNPSLKSRISFTRDTSKNQFFLQLTSVTTEDTATYYCARLDFGNYGGAMDYWGQGTSVTVSS

SEQ ID NO: 2 - protein, 107 aa, Artificial Sequence
  900424 VL
DIVMTQSHKFMSTSIGDRVSITCKASQHVSTAVAWYQQKPGQSPKLLIYSASYRYTGVPDRFTGSRSGTDFTFTISSVQAEDLAVYYCQQHYITPYTFGGGTKLEIK

SEQ ID NO: 3 - protein, 9 aa, Artificial Sequence
  HCDR1
GYSITSDYA

SEQ ID NO: 4 - protein, 7 aa, Artificial Sequence
  HCDR2
ITSSGST

SEQ ID NO: 5 - protein, 14 aa, Artificial Sequence
  HCDR3
ARLDFGNYGGAMDY

SEQ ID NO: 6 - protein, 6 aa, Artificial Sequence
  LCDR1
QHVSTA

SEQ ID NO: 7 - protein, 3 aa, Artificial Sequence
  LCDR2
SAS

SEQ ID NO: 8 - protein, 9 aa, Artificial Sequence
  LCDR3
QQHYITPYT

SEQ ID NO: 9 - protein, 121 aa, Artificial Sequence
  VH of HB0030 and HB0031
QVQLQESGPGLVKPSETLSLTCTVSGYSITSDYAWIWIRQPPGKGLEWIGYITSSGSTYYNPSLKSRVTFSVDTSKNQFSLKLSSVTAADTATYYCARLDFGNYGGAMDYWGQGTLVTVSS

SEQ ID NO: 10 - protein, 107 aa, Artificial Sequence
  HB0030 VL
DIQMTQSPSSLSASVGDRVTITCRASQHVSTAVNWYQQKPGKAPKLLIYSASYLYSGVPSRFSGSRSGTDFTLTISSLQPEDFATYYCQQHYITPYTFGQGTKLEIK

SEQ ID NO: 11 - protein, 107 aa, Artificial Sequence
  VL of HB0031 and HB0033
DIQMTQSPSSLSASVGDRVTITCKASQHVSTALAWYQQKPGKAPKLLIYSASYLQSGVPSRFSGSRSGTDFTLTISSLQPEDFATYYCQQHYITPYTFGQGTKLEIK

SEQ ID NO: 12 - protein, 121 aa, Artificial Sequence
  HB0032 VH
QVQLQESGPGLVKPSETLSLTCTVSGYSITSDYAWIWIRQPPGKKLEWIGYITSSGSTYYNPSLKSRVTFSVDTSKNQFSLKLSSVTAADTATYYCARLDFGNYGGAMDYWGQGTLVTVSS

SEQ ID NO: 13 - protein, 107 aa, Artificial Sequence
  HB0032 VL
DIQMTQSPSSLSASVGDRVTITCKASQHVSTAVNWYQQKPGKAPKLLIYSASYRQSGVPSRFSGSGSGTDFTLTISSLQPEDFATYYCQQHYITPYTFGQGTKLEIK

SEQ ID NO: 14 - protein, 121 aa, Artificial Sequence
  HB0033 VH
QVQLQESGPGLVKPSETLSLTCTVSGYSITSDYAWIWIRQPPGNKLEWIGYITSSGSTYYNPSLKSRVTFSVDTSKNQFSLKLSSVTAADTATYYCARLDFGNYGGAMDYWGQGTLVTVSS

SEQ ID NO: 15 - protein, 26 aa, Artificial Sequence [sequence omitted]

SEQ ID NO: 16 - protein, 26 aa, Artificial Sequence [sequence omitted]

SEQ ID NO: 17 - protein, 17 aa, Artificial Sequence
  L-FR2 of HB0030 and HB0032
VNWYQQKPGKAPKLLIY

SEQ ID NO: 18 - protein, 17 aa, Artificial Sequence
  L-FR2 of HB0031 and HB0033
LAWYQQKPGKAPKLLIY

SEQ ID NO: 19 - protein, 36 aa, Artificial Sequence
  HB0030 L-FR3
YLYSGVPSRFSGSRSGTDFTLTISSLQPEDFATYYC

SEQ ID NO: 20 - protein, 36 aa, Artificial Sequence
  L-FR3 of HB0031 and HB0033
YLQSGVPSRFSGSRSGTDFTLTISSLQPEDFATYYC

SEQ ID NO: 21 - protein, 36 aa, Artificial Sequence
  HB0032 L-FR3
YRQSGVPSRFSGSGSGTDFTLTISSLQPEDFATYYC

SEQ ID NO: 22 - protein, 10 aa, Artificial Sequence
  L-FR4 of HB0030 HB0031 HB0032 and HB0033
FGQGTKLEIK

SEQ ID NO: 23 - protein, 25 aa, Artificial Sequence
  H-FR1 of HB0030 HB0031 HB0032 and HB0033
QVQLQESGPGLVKPSETLSLTCTVS

SEQ ID NO: 24 - protein, 17 aa, Artificial Sequence
  H-FR2 of HB0030 and HB0031
WIWIRQPPGKGLEWIGY

SEQ ID NO: 25 - protein, 17 aa, Artificial Sequence
  HB0032 H-FR2
WIWIRQPPGKKLEWIGY

SEQ ID NO: 26 - protein, 17 aa, Artificial Sequence
  HB0033 H-FR2
WIWIRQPPGNKLEWIGY

SEQ ID NO: 27 - protein, 38 aa, Artificial Sequence
  H-FR3 of HB0030 HB0031 HB0032 and HB0033
YYNPSLKSRVTFSVDTSKNQFSLKLSSVTAADTATYYC

SEQ ID NO: 28 - protein, 11 aa, Artificial Sequence
  H-FR4 of HB0030 HB0031 HB0032 and HB0033
WGQGTLVTVSS

SEQ ID NO: 29 - protein, 329 aa, Artificial Sequence
  Human IgG1 constant region wild type
ASTKGPSVFPLAPSSKSTSGGTAALGCLVKDYFPEPVTVSWNSGALTSGVHTFPAVLQSSGLYSLSSVVTVPSSSLGTQTYICNVNHKPSNTKVDKRVEPKSCDKTHTCPPCPAPELLGGPSVFLFPPKPKDTLMISRTPEVTCVVVDVSHEDPEVKFNWYVDGVEVHNAKTKPREEQYNSTYRVVSVLTVLHQDWLNGKEYKCKVSNKALPAPIEKTISKAKGQPREPQVYTLPPSREEMTKNQVSLTCLVKGFYPSDIAVEWESNGQPENNYKTTPPVLDSDGSFFLYSKLTVDKSRWQQGNVFSCSVMHEALHNHYTQKSLSLSPG

SEQ ID NO: 30 - protein, 329 aa, Artificial Sequence
  Human IgG1 constant region mutation
ASTKGPSVFPLAPSSKSTSGGTAALGCLVKDYFPEPVTVSWNSGALTSGVHTFPAVLQSSGLYSLSSVVTVPSSSLGTQTYICNVNHKPSNTKVDKRVEPKSCDKTHTCPPCPAPEAAGGPSVFLFPPKPKDTLMISRTPEVTCVVVDVSHEDPEVKFNWYVDGVEVHNAKTKPREEQYNSTYRVVSVLTVLHQDWLNGKEYKCKVSNKALPAPIEKTISKAKGQPREPQVYTLPPSREEMTKNQVSLTCLVKGFYPSDIAVEWESNGQPENNYKTTPPVLDSDGSFFLYSKLTVDKSRWQQGNVFSCSVMHEALHNHYTQKSLSLSPG

SEQ ID NO: 31 - protein, 107 aa, Artificial Sequence [sequence omitted]

SEQ ID NO: 32 - protein, 119 aa, Artificial Sequence
  VH of 900423 and 900428VH
DVQLQESGPGLVKPSQSLSLTCTVTGYSITSDYAWNWIRQFPGNRLEWMGYISYSGAPRYNPSLKSRISITRDTSKNQFFLQLSFVTTEDTATYYCASLGTDYYAMDYWGQGTSVIVSS

SEQ ID NO: 33 - protein, 107 aa, Artificial Sequence
  900428VL
DIVMTQSHKFMFTSVGDRVSITCKASQHVSNAVAWYQQKPGQSPKLLIHSASYRYTGVPDRFTGRGSGTDFTFTINSVQAEDLAVYYCQQYYSLPWTFGGGTKLEIK

SEQ ID NO: 34 - protein, 107 aa, Artificial Sequence
  900423VL
DIVMTQSHKFMFTSVGDRVSITCKASQHVSNAVAWYQQKPGQSPKLLIHSASYRYTGVPDRFIGRGSGTDFTFTISSVQAEDLAVYYCQQYYSLPWTFGGGTKLEIK

SEQ ID NO: 35 - protein, 25 aa, Artificial Sequence
  H-FR1 of 900423 900424 and 900428
DVQLQESGPGLVKPSQSLSLTCTVT

SEQ ID NO: 36 - protein, 17 aa, Artificial Sequence
  900424 H-FR2
WIWIRQFPGNKVEWMGY

SEQ ID NO: 37 - protein, 17 aa, Artificial Sequence
  H-FR2 of 900423 and 900428
WNWIRQFPGNRLEWMGY

SEQ ID NO: 38 - protein, 38 aa, Artificial Sequence
  900424 H-FR3
SYNPSLKSRISFTRDTSKNQFFLQLTSVTTEDTATYYC

SEQ ID NO: 39 - protein, 38 aa, Artificial Sequence
  H-FR3 of 900423 and 900428
RYNPSLKSRISITRDTSKNQFFLQLSFVTTEDTATYYC

SEQ ID NO: 40 - protein, 11 aa, Artificial Sequence
  900424 H-FR4
WGQGTSVTVSS

SEQ ID NO: 41 - protein, 11 aa, Artificial Sequence
  H-FR4 of 900423 and 900428
WGQGTSVIVSS

SEQ ID NO: 42 - protein, 7 aa, Artificial Sequence
  HCDR2 of 900423 and 900428
ISYSGAP

SEQ ID NO: 43 - protein, 12 aa, Artificial Sequence
  HCDR3 of 900423 and 900428
ASLGTDYYAMDY

SEQ ID NO: 44 - protein, 26 aa, Artificial Sequence
  900424 L-FR1
DIVMTQSHKFMSTSIGDRVSITCKAS

SEQ ID NO: 45 - protein, 26 aa, Artificial Sequence
  L-FR1 of 900423 and 900428
DIVMTQSHKFMFTSVGDRVSITCKAS

SEQ ID NO: 46 - protein, 17 aa, Artificial Sequence
  900424 L-FR2
VAWYQQKPGQSPKLLIY

SEQ ID NO: 47 - protein, 17 aa, Artificial Sequence
  L-FR2 of 900423 and 900428
VAWYQQKPGQSPKLLIH

SEQ ID NO: 48 - protein, 36 aa, Artificial Sequence
  900428 L-FR3
YRYTGVPDRFTGRGSGTDFTFTINSVQAEDLAVYYC

SEQ ID NO: 49 - protein, 36 aa, Artificial Sequence
  900424 L-FR3
YRYTGVPDRFTGSRSGTDFTFTISSVQAEDLAVYYC

SEQ ID NO: 50 - protein, 36 aa, Artificial Sequence
  900423 L-FR3
YRYTGVPDRFIGRGSGTDFTFTISSVQAEDLAVYYC

SEQ ID NO: 51 - protein, 10 aa, Artificial Sequence
  L-FR4 of 900423 900424 and 900428
FGGGTKLEIK

SEQ ID NO: 52 - protein, 6 aa, Artificial Sequence
  LCDR1 of 900423 and 900428
QHVSNA

SEQ ID NO: 53 - protein, 9 aa, Artificial Sequence
  LCDR3 of 900423 and 900428
QQYYSLPWT

SEQ ID NO: 54 - protein, 121 aa, Artificial Sequence
  VH of HB0030 and HB0031; HB0032 VH;HB0033 VH
  misc_feature (44)..(44): Xaa = Lys or Asn
  misc_feature (45)..(45): Xaa = Gly or Lys
QVQLQESGPGLVKPSETLSLTCTVSGYSITSDYAWIWIRQPPGXXLEWIGYITSSGSTYYNPSLKSRVTFSVDTSKNQFSLKLSSVTAADTATYYCARLDFGNYGGAMDYWGQGTLVTVSS

SEQ ID NO: 55 - protein, 121 aa, Artificial Sequence
  900424 VH; HB0030 and HB0031 VH; HB0032 VH; HB0033 VH; 900423 and 900428VH
  misc_feature (1)..(1): Xaa = Asp or Gln
  misc_feature (16)..(16): Xaa = Glu or Gln
  misc_feature (17)..(17): Xaa = Ser or Thr
  misc_feature (25)..(25): Xaa = Ser or Thr
  misc_feature (36)..(36): Xaa = Ile or Asn
  misc_feature (41)..(41): Xaa = Phe or Pro
  misc_feature (44)..(44): Xaa = Lys or Asn
  misc_feature (45)..(45): Xaa = Gly Lys or Arg
  misc_feature (46)..(46): Xaa = Leu or Val
  misc_feature (49)..(49): Xaa = Ile or Met
  misc_feature (53)..(53): Xaa = Ser or Thr
  misc_feature (54)..(54): Xaa = Ser or Tyr
  misc_feature (57)..(57): Xaa = Ala or Ser
  misc_feature (58)..(58): Xaa = Pro or Thr
  misc_feature (59)..(59): Xaa = Arg Ser or Tyr
  misc_feature (68)..(68): Xaa = Ile or Val
  misc_feature (69)..(69): Xaa = Ser or Thr
  misc_feature (70)..(70): Xaa = Phe or Ile
  misc_feature (71)..(71): Xaa = Ser or Thr
  misc_feature (72)..(72): Xaa = Arg or Val
  misc_feature (80)..(80): Xaa = Phe or Ser
  misc_feature (82)..(82): Xaa = Lys or Gln
  misc_feature (84)..(84): Xaa = Ser or Thr
  misc_feature (85)..(85): Xaa = Phe or Ser
  misc_feature (88)..(88): Xaa = Ala or Thr
  misc_feature (89)..(89): Xaa = Ala or Glu
  misc_feature (98)..(98): Xaa = Arg or Ser
  misc_feature (100)..(100): Xaa = Asp or Gly
  misc_feature (101)..(101): Xaa = Phe or Thr
  misc_feature (102)..(102): Xaa = Asp or Gly
  misc_feature (103)..(103): Xaa = Asn or Tyr
  misc_feature (105)..(105): Xaa = Gly or absent
  misc_feature (106)..(106): Xaa = Gly or absent
  misc_feature (116)..(116): Xaa = Leu or Ser
  misc_feature (118)..(118): Xaa = Ile or Thr
XVQLQESGPGLVKPSXXLSLTCTVXGYSITSDYAWXWIRQXPGXXXEWXGYIXXSGXXXYNPSLKSRXXXXXDTSKNQFXLXLXXVTXXDTATYYCAXLXXXXYXXAMDYWGQGTXVXVSS

SEQ ID NO: 56 - protein, 7 aa, Artificial Sequence
  HCDR2 of 900424 HB0030 HB0031 HB0032 and HB0033;HCDR2 of 900423 and 900428
  misc_feature (2)..(2): Xaa = Ser or Thr
  misc_feature (3)..(3): Xaa = Ser or Tyr
  misc_feature (6)..(6): Xaa = Ala or Ser
  misc_feature (7)..(7): Xaa = Pro or Thr
IXXSGXX

SEQ ID NO: 57 - protein, 14 aa, Artificial Sequence
  HCDR3 of 900423 and 900428; HCDR3 of 900424 HB0030 HB0031 HB0032 and HB0033
  misc_feature (2)..(2): Xaa = Arg or Ser
  misc_feature (4)..(4): Xaa = Asp or Gly
  misc_feature (5)..(5): Xaa = Phe or Thr
  misc_feature (6)..(6): Xaa = Asp or Gly
  misc_feature (7)..(7): Xaa = Asn or Tyr
  misc_feature (9)..(9): Xaa = Gly or absent
  misc_feature (10)..(10): Xaa = Gly or absent
AXLXXXXYXXAMDY

SEQ ID NO: 58 - protein, 25 aa, Artificial Sequence
  H-FR1 of HB0030 HB0031 HB0032 and HB0033; H-FR1 of 900423 900424 and 900428
  misc_feature (1)..(1): Xaa = Asp or Gln
  misc_feature (16)..(16): Xaa = Glu or Gln
  misc_feature (17)..(17): Xaa = Ser or Thr
  misc_feature (25)..(25): Xaa = Ser or Thr
XVQLQESGPGLVKPSXXLSLTCTVX

SEQ ID NO: 59 - protein, 17 aa, Artificial Sequence
  H-FR2 of HB0030 and HB0031 ; HB0032 H-FR2; HB0033 H-FR2
  misc_feature (10)..(10): Xaa = Lys or Asn
  misc_feature (11)..(11): Xaa = Gly or Lys
WIWIRQPPGXXLEWIGY

SEQ ID NO: 60 - protein, 17 aa, Artificial Sequence
  H-FR2 of HB0030 and HB0031; HB0032 H-FR2; HB0033 H-FR2; 900424 H-FR2; H-FR2 of 900423 and 900428
  misc_feature (2)..(2): Xaa = Ile or Asn
  misc_feature (7)..(7): Xaa = Phe or Pro
  misc_feature (10)..(10): Xaa = Lys or Asn
  misc_feature (11)..(11): Xaa = Gly Lys or Arg
  misc_feature (12)..(12): Xaa = Leu or Val
  misc_feature (15)..(15): Xaa = Ile or Met
WXWIRQXPGXXXEWXGY

SEQ ID NO: 61 - protein, 38 aa, Artificial Sequence
  H-FR3 of HB0030 HB0031 HB0032 and HB0033; H-FR3 of 900423 and 900428; 900424 H-FR3
  misc_feature (1)..(1): Xaa = Arg Ser or Tyr
  misc_feature (10)..(10): Xaa = Ile or Val
  misc_feature (11)..(11): Xaa = Ser or Thr
  misc_feature (12)..(12): Xaa = Phe or Ile
  misc_feature (13)..(13): Xaa = Ser or Thr
  misc_feature (14)..(14): Xaa = Arg or Val
  misc_feature (22)..(22): Xaa = Phe or Ser
  misc_feature (24)..(24): Xaa = Lys or Gln
  misc_feature (26)..(26): Xaa = Ser or Thr
  misc_feature (27)..(27): Xaa = Phe or Ser
  misc_feature (30)..(30): Xaa = Ala or Thr
  misc_feature (31)..(31): Xaa = Ala or Glu
XYNPSLKSRXXXXXDTSKNQFXLXLXXVTXXDTATYYC

SEQ ID NO: 62 - protein, 11 aa, Artificial Sequence
  H-FR4 of HB0030 HB0031 HB0032 and HB0033 H-FR4; 900424 H-FR4; H-FR4 of 900423 and 900428
  misc_feature (6)..(6): Xaa = Leu or Ser
  misc_feature (8)..(8): Xaa = Ile or Thr
WGQGTXVXVSS

SEQ ID NO: 63 - protein, 107 aa, Artificial Sequence
  HB0030 VL; VL of HB0031 and HB0033 ; HB0032 VL
  misc_feature (24)..(24): Xaa = Lys or Arg
  misc_feature (33)..(33): Xaa = Leu or Val
  misc_feature (34)..(34): Xaa = Ala or Asn
  misc_feature (54)..(54): Xaa = Leu or Arg
  misc_feature (55)..(55): Xaa = Gln or Tyr
  misc_feature (66)..(66): Xaa = Gly or Arg
DIQMTQSPSSLSASVGDRVTITCXASQHVSTAXXWYQQKPGKAPKLLIYSASYXXSGVPSRFSGSXSGTDFTLTISSLQPEDFATYYCQQHYITPYTFGQGTKLEIK

SEQ ID NO: 64 - protein, 107 aa, Artificial Sequence
  900424 VL; HB0030 VL; VL of HB0031 and HB0033; HB0032 VL; 900423VL; 900428VL
  misc_feature (3)..(3): Xaa = Gln or Val
  misc_feature (8)..(8): Xaa = His or Pro
  misc_feature (9)..(9): Xaa = Lys or Ser
  misc_feature (10)..(10): Xaa = Phe or Ser
  misc_feature (11)..(11): Xaa = Leu or Met
  misc_feature (12)..(12): Xaa = Phe or Ser
  misc_feature (13)..(13): Xaa = Ala or Thr
  misc_feature (15)..(15): Xaa = Ile or Val
  misc_feature (20)..(20): Xaa = Ser or Thr
  misc_feature (24)..(24): Xaa = Lys or Arg
  misc_feature (31)..(31): Xaa = Asn or Thr
  misc_feature (33)..(33): Xaa = Leu or Val
  misc_feature (34)..(34): Xaa = Ala or Asn
  misc_feature (42)..(42): Xaa = Lys or Gln
  misc_feature (43)..(43): Xaa = Ala or Ser
  misc_feature (49)..(49): Xaa = His or Tyr
  misc_feature (54)..(54): Xaa = Leu or Arg
  misc_feature (55)..(55): Xaa = Gln or Tyr
  misc_feature (56)..(56): Xaa = Ser or Thr
  misc_feature (60)..(60): Xaa = Asp or Ser
  misc_feature (63)..(63): Xaa = Ile Ser or Thr
  misc_feature (65)..(65): Xaa = Arg or Ser
  misc_feature (66)..(66): Xaa = Gly or Arg
  misc_feature (73)..(73): Xaa = Phe or Leu
  misc_feature (76)..(76): Xaa = Asn or Ser
  misc_feature (78)..(78): Xaa = Leu or Val
  misc_feature (80)..(80): Xaa = Ala or Pro
  misc_feature (83)..(83): Xaa = Phe or Leu
  misc_feature (85)..(85): Xaa = Thr or Val
  misc_feature (91)..(91): Xaa = His or Tyr
  misc_feature (93)..(93): Xaa = Ile or Ser
  misc_feature (94)..(94): Xaa = Leu or Thr
  misc_feature (96)..(96): Xaa = Trp or Tyr
  misc_feature (100)..(100): Xaa = Gly or Gln
DIXMTQSXXXXXXSXGDRVXITCXASQHVSXAXXWYQQKPGXXPKLLIXSASYXXXGVPXRFXGXXSGTDFTXTIXSXQXEDXAXYYCQQXYXXPXTFGXGTKLEIK

SEQ ID NO: 65 - protein, 6 aa, Artificial Sequence
  LCDR1 of 900424 HB0030 HB0031 HB0032 and HB0033;LCDR1 of 900423 and 900428
  misc_feature (5)..(5): Xaa = Asn or Thr
QHVSXA

SEQ ID NO: 66 - protein, 9 aa, Artificial Sequence
  LCDR3 of 900424 HB0030 HB0031 HB0032 and HB0033; LCDR3 of 900423 and 900428
  misc_feature (3)..(3): Xaa = His or Tyr
  misc_feature (5)..(5): Xaa = Ile or Ser
  misc_feature (6)..(6): Xaa = Leu or Thr
  misc_feature (8)..(8): Xaa = Trp or Tyr
QQXYXXPXT

SEQ ID NO: 67 - protein, 26 aa, Artificial Sequence
  L-FR1 of HB0031 HB0032 and HB0033; HB0030 L-FR1
  misc_feature (24)..(24): Xaa = Lys or Arg
DIQMTQSPSSLSASVGDRVTITCXAS

SEQ ID NO: 68 - protein, 26 aa, Artificial Sequence
  HB0030 L-FR1; L-FR1 of HB0031 HB0032 and HB0033 L-FR1; 900424 L-FR1; L-FR1 of 900423 and 900428
  misc_feature (3)..(3): Xaa = Gln or Val
  misc_feature (8)..(8): Xaa = His or Pro
  misc_feature (9)..(9): Xaa = Lys or Ser
  misc_feature (10)..(10): Xaa = Phe or Ser
  misc_feature (11)..(11): Xaa = Leu or Met
  misc_feature (12)..(12): Xaa = Phe or Ser
  misc_feature (13)..(13): Xaa = Ala or Thr
  misc_feature (15)..(15): Xaa = Ile or Val
  misc_feature (20)..(20): Xaa = Ser or Thr
  misc_feature (24)..(24): Xaa = Lys or Arg
DIXMTQSXXXXXXSXGDRVXITCXAS

SEQ ID NO: 69 - protein, 17 aa, Artificial Sequence
  L-FR2 of HB0030 and HB0032 L-FR2; L-FR2 of HB0031 and HB0033
  misc_feature (1)..(1): Xaa = Leu or Val
  misc_feature (2)..(2): Xaa = Ala or Asn
XXWYQQKPGKAPKLLIY

SEQ ID NO: 70 - protein, 17 aa, Artificial Sequence
  L-FR2 of HB0030 and HB0032;  L-FR2 of HB0031 and HB0033; 900424 L-FR2; L-FR2 of 900423 and 900428
  misc_feature (1)..(1): Xaa = Leu or Val
  misc_feature (2)..(2): Xaa = Ala or Asn
  misc_feature (10)..(10): Xaa = Lys or Gln
  misc_feature (11)..(11): Xaa = Ala or Ser
  misc_feature (17)..(17): Xaa = His or Tyr
XXWYQQKPGXXPKLLIX

SEQ ID NO: 71 - protein, 36 aa, Artificial Sequence
  HB0030 L-FR3; L-FR3 of HB0031 and HB0033 ; HB0032 L-FR3
  misc_feature (2)..(2): Xaa = Leu or Arg
  misc_feature (3)..(3): Xaa = Gln or Tyr
  misc_feature (14)..(14): Xaa = Gly or Arg
YXXSGVPSRFSGSXSGTDFTLTISSLQPEDFATYYC

SEQ ID NO: 72 - protein, 36 aa, Artificial Sequence
  HB0030 L-FR3; L-FR3 of HB0031 and HB0033; HB0032 L-FR3; 900428 L-FR3; 900424 L-FR3; 900423 L-FR3
  misc_feature (2)..(2): Xaa = Leu or Arg
  misc_feature (3)..(3): Xaa = Gln or Tyr
  misc_feature (4)..(4): Xaa = Ser or Thr
  misc_feature (8)..(8): Xaa = Asp or Ser
  misc_feature (11)..(11): Xaa = Ile Ser or Thr
  misc_feature (13)..(13): Xaa = Arg or Ser
  misc_feature (14)..(14): Xaa = Gly or Arg
  misc_feature (21)..(21): Xaa = Phe or Leu
  misc_feature (24)..(24): Xaa = Asn or Ser
  misc_feature (26)..(26): Xaa = Leu or Val
  misc_feature (28)..(28): Xaa = Ala or Pro
  misc_feature (31)..(31): Xaa = Phe or Leu
  misc_feature (33)..(33): Xaa = Thr or Val
YXXXGVPXRFXGXXSGTDFTXTIXSXQXEDXAXYYC

SEQ ID NO: 73 - protein, 10 aa, Artificial Sequence
  L-FR4 of 900423 900424 and 900428 ; L-FR4 of HB0030 HB0031 HB0032 and HB0033
  misc_feature (3)..(3): Xaa = Gly or Gln
FGXGTKLEIK

SEQ ID NO: 74 - protein, 15 aa, Artificial Sequence
  Linker1
GGGGSGGGGSGGGGS

SEQ ID NO: 75 - protein, 20 aa, Artificial Sequence
  Linker2
GGGGSGGGGSGGGGSGGGGS

SEQ ID NO: 76 - protein, 25 aa, Artificial Sequence
  Linker3
GGGGSGGGGSGGGGSGGGGSGGGGS

SEQ ID NO: 77 - protein, 30 aa, Artificial Sequence
  Linker4
GGGGSGGGGSGGGGSGGGGSGGGGSGGGGS

SEQ ID NO: 78 - protein, 717 aa, Artificial Sequence
  900681 heavy chain
QVQLQESGPGLVKPSETLSLTCTVSGYSITSDYAWIWIRQPPGKGLEWIGYITSSGSTYYNPSLKSRVTFSVDTSKNQFSLKLSSVTAADTATYYCARLDFGNYGGAMDYWGQGTLVTVSSASTKGPSVFPLAPSSKSTSGGTAALGCLVKDYFPEPVTVSWNSGALTSGVHTFPAVLQSSGLYSLSSVVTVPSSSLGTQTYICNVNHKPSNTKVDKRVEPKSCDKTHTCPPCPAPELLGGPSVFLFPPKPKDTLMISRTPEVTCVVVDVSHEDPEVKFNWYVDGVEVHNAKTKPREEQYNSTYRVVSVLTVLHQDWLNGKEYKCKVSNKALPAPIEKTISKAKGQPREPQVYTLPPSREEMTKNQVSLTCLVKGFYPSDIAVEWESNGQPENNYKTTPPVLDSDGSFFLYSKLTVDKSRWQQGNVFSCSVMHEALHNHYTQKSLSLSPGGGGGSGGGGSGGGGSGGGGSDVVMTQTPLSLSVTPGQPASISCKSSQSLANSYGNTYLSWYLHKPGQSPQLLIYGISNRFSGVPDRFSGSGSGTDFTLKISRVEAEDVGVYYCLQGTHQPPTFGCGTKLEIKGGGGSGGGGSGGGGSQVQLVQSGAEVKKPGASVKVSCKASGYAFTGYTIHWVRQAPGQCLEWMGWFYPGSGTLKYSEKFQGRVTITRDKSLSTAYMELSSLRSEDTAVYYCARHGTGTLMAMDYWGQGTLVTVSS

SEQ ID NO: 79 - protein, 722 aa, Artificial Sequence
  900683 heavy chain
QVQLQESGPGLVKPSETLSLTCTVSGYSITSDYAWIWIRQPPGKGLEWIGYITSSGSTYYNPSLKSRVTFSVDTSKNQFSLKLSSVTAADTATYYCARLDFGNYGGAMDYWGQGTLVTVSSASTKGPSVFPLAPSSKSTSGGTAALGCLVKDYFPEPVTVSWNSGALTSGVHTFPAVLQSSGLYSLSSVVTVPSSSLGTQTYICNVNHKPSNTKVDKRVEPKSCDKTHTCPPCPAPELLGGPSVFLFPPKPKDTLMISRTPEVTCVVVDVSHEDPEVKFNWYVDGVEVHNAKTKPREEQYNSTYRVVSVLTVLHQDWLNGKEYKCKVSNKALPAPIEKTISKAKGQPREPQVYTLPPSREEMTKNQVSLTCLVKGFYPSDIAVEWESNGQPENNYKTTPPVLDSDGSFFLYSKLTVDKSRWQQGNVFSCSVMHEALHNHYTQKSLSLSPGGGGGSGGGGSGGGGSGGGGSDVVMTQTPLSLSVTPGQPASISCKSSQSLANSYGNTYLSWYLHKPGQSPQLLIYGISNRFSGVPDRFSGSGSGTDFTLKISRVEAEDVGVYYCLQGTHQPPTFGQGTKLEIKGGGGSGGGGSGGGGSGGGGSQVQLVQSGAEVKKPGASVKVSCKASGYAFTGYTIHWVRQAPGQRLEWMGWFYPGSGTLKYSEKFQGRVTITRDKSLSTAYMELSSLRSEDTAVYYCARHGTGTLMAMDYWGQGTLVTVSS

SEQ ID NO: 80 - protein, 727 aa, Artificial Sequence
  900684 heavy chain
QVQLQESGPGLVKPSETLSLTCTVSGYSITSDYAWIWIRQPPGKGLEWIGYITSSGSTYYNPSLKSRVTFSVDTSKNQFSLKLSSVTAADTATYYCARLDFGNYGGAMDYWGQGTLVTVSSASTKGPSVFPLAPSSKSTSGGTAALGCLVKDYFPEPVTVSWNSGALTSGVHTFPAVLQSSGLYSLSSVVTVPSSSLGTQTYICNVNHKPSNTKVDKRVEPKSCDKTHTCPPCPAPELLGGPSVFLFPPKPKDTLMISRTPEVTCVVVDVSHEDPEVKFNWYVDGVEVHNAKTKPREEQYNSTYRVVSVLTVLHQDWLNGKEYKCKVSNKALPAPIEKTISKAKGQPREPQVYTLPPSREEMTKNQVSLTCLVKGFYPSDIAVEWESNGQPENNYKTTPPVLDSDGSFFLYSKLTVDKSRWQQGNVFSCSVMHEALHNHYTQKSLSLSPGGGGGSGGGGSGGGGSGGGGSDVVMTQTPLSLSVTPGQPASISCKSSQSLANSYGNTYLSWYLHKPGQSPQLLIYGISNRFSGVPDRFSGSGSGTDFTLKISRVEAEDVGVYYCLQGTHQPPTFGQGTKLEIKGGGGSGGGGSGGGGSGGGGSGGGGSQVQLVQSGAEVKKPGASVKVSCKASGYAFTGYTIHWVRQAPGQRLEWMGWFYPGSGTLKYSEKFQGRVTITRDKSLSTAYMELSSLRSEDTAVYYCARHGTGTLMAMDYWGQGTLVTVSS

SEQ ID NO: 81 - protein, 727 aa, Artificial Sequence
  900685 heavy chain
QVQLQESGPGLVKPSETLSLTCTVSGYSITSDYAWIWIRQPPGKGLEWIGYITSSGSTYYNPSLKSRVTFSVDTSKNQFSLKLSSVTAADTATYYCARLDFGNYGGAMDYWGQGTLVTVSSASTKGPSVFPLAPSSKSTSGGTAALGCLVKDYFPEPVTVSWNSGALTSGVHTFPAVLQSSGLYSLSSVVTVPSSSLGTQTYICNVNHKPSNTKVDKRVEPKSCDKTHTCPPCPAPELLGGPSVFLFPPKPKDTLMISRTPEVTCVVVDVSHEDPEVKFNWYVDGVEVHNAKTKPREEQYNSTYRVVSVLTVLHQDWLNGKEYKCKVSNKALPAPIEKTISKAKGQPREPQVYTLPPSREEMTKNQVSLTCLVKGFYPSDIAVEWESNGQPENNYKTTPPVLDSDGSFFLYSKLTVDKSRWQQGNVFSCSVMHEALHNHYTQKSLSLSPGGGGGSGGGGSGGGGSGGGGSDVVMTQTPLSLSVTPGQPASISCKSSQSLANSYGNTYLSWYLHKPGQSPQLLIYGISNRFSGVPDRFSGSGSGTDFTLKISRVEAEDVGVYYCLQGTHQPPTFGCGTKLEIKGGGGSGGGGSGGGGSGGGGSGGGGSQVQLVQSGAEVKKPGASVKVSCKASGYAFTGYTIHWVRQAPGQCLEWMGWFYPGSGTLKYSEKFQGRVTITRDKSLSTAYMELSSLRSEDTAVYYCARHGTGTLMAMDYWGQGTLVTVSS

SEQ ID NO: 82 - protein, 732 aa, Artificial Sequence
  900686 heavy chain
QVQLQESGPGLVKPSETLSLTCTVSGYSITSDYAWIWIRQPPGKGLEWIGYITSSGSTYYNPSLKSRVTFSVDTSKNQFSLKLSSVTAADTATYYCARLDFGNYGGAMDYWGQGTLVTVSSASTKGPSVFPLAPSSKSTSGGTAALGCLVKDYFPEPVTVSWNSGALTSGVHTFPAVLQSSGLYSLSSVVTVPSSSLGTQTYICNVNHKPSNTKVDKRVEPKSCDKTHTCPPCPAPELLGGPSVFLFPPKPKDTLMISRTPEVTCVVVDVSHEDPEVKFNWYVDGVEVHNAKTKPREEQYNSTYRVVSVLTVLHQDWLNGKEYKCKVSNKALPAPIEKTISKAKGQPREPQVYTLPPSREEMTKNQVSLTCLVKGFYPSDIAVEWESNGQPENNYKTTPPVLDSDGSFFLYSKLTVDKSRWQQGNVFSCSVMHEALHNHYTQKSLSLSPGGGGGSGGGGSGGGGSGGGGSDVVMTQTPLSLSVTPGQPASISCKSSQSLANSYGNTYLSWYLHKPGQSPQLLIYGISNRFSGVPDRFSGSGSGTDFTLKISRVEAEDVGVYYCLQGTHQPPTFGQGTKLEIKGGGGSGGGGSGGGGSGGGGSGGGGSGGGGSQVQLVQSGAEVKKPGASVKVSCKASGYAFTGYTIHWVRQAPGQRLEWMGWFYPGSGTLKYSEKFQGRVTITRDKSLSTAYMELSSLRSEDTAVYYCARHGTGTLMAMDYWGQGTLVTVSS

SEQ ID NO: 83 - protein, 732 aa, Artificial Sequence
  900687 heavy chain
QVQLQESGPGLVKPSETLSLTCTVSGYSITSDYAWIWIRQPPGKGLEWIGYITSSGSTYYNPSLKSRVTFSVDTSKNQFSLKLSSVTAADTATYYCARLDFGNYGGAMDYWGQGTLVTVSSASTKGPSVFPLAPSSKSTSGGTAALGCLVKDYFPEPVTVSWNSGALTSGVHTFPAVLQSSGLYSLSSVVTVPSSSLGTQTYICNVNHKPSNTKVDKRVEPKSCDKTHTCPPCPAPELLGGPSVFLFPPKPKDTLMISRTPEVTCVVVDVSHEDPEVKFNWYVDGVEVHNAKTKPREEQYNSTYRVVSVLTVLHQDWLNGKEYKCKVSNKALPAPIEKTISKAKGQPREPQVYTLPPSREEMTKNQVSLTCLVKGFYPSDIAVEWESNGQPENNYKTTPPVLDSDGSFFLYSKLTVDKSRWQQGNVFSCSVMHEALHNHYTQKSLSLSPGGGGGSGGGGSGGGGSGGGGSDVVMTQTPLSLSVTPGQPASISCKSSQSLANSYGNTYLSWYLHKPGQSPQLLIYGISNRFSGVPDRFSGSGSGTDFTLKISRVEAEDVGVYYCLQGTHQPPTFGCGTKLEIKGGGGSGGGGSGGGGSGGGGSGGGGSGGGGSQVQLVQSGAEVKKPGASVKVSCKASGYAFTGYTIHWVRQAPGQCLEWMGWFYPGSGTLKYSEKFQGRVTITRDKSLSTAYMELSSLRSEDTAVYYCARHGTGTLMAMDYWGQGTLVTVSS

SEQ ID NO: 84 - protein, 214 aa, Artificial Sequence
  HB0030 heavy chain
DIQMTQSPSSLSASVGDRVTITCRASQHVSTAVNWYQQKPGKAPKLLIYSASYLYSGVPSRFSGSRSGTDFTLTISSLQPEDFATYYCQQHYITPYTFGQGTKLEIKRTVAAPSVFIFPPSDEQLKSGTASVVCLLNNFYPREAKVQWKVDNALQSGNSQESVTEQDSKDSTYSLSSTLTLSKADYEKHKVYACEVTHQGLSSPVTKSFNRGEC

SEQ ID NO: 85 - protein, 712 aa, Artificial Sequence
  900691 heavy chain
QVQLVQSGAEVKKPGASVKVSCKASGYAFTGYTIHWVRQAPGQRLEWMGWFYPGSGTLKYSEKFQGRVTITRDKSLSTAYMELSSLRSEDTAVYYCARHGTGTLMAMDYWGQGTLVTVSSASTKGPSVFPLAPSSKSTSGGTAALGCLVKDYFPEPVTVSWNSGALTSGVHTFPAVLQSSGLYSLSSVVTVPSSSLGTQTYICNVNHKPSNTKVDKRVEPKSCDKTHTCPPCPAPELLGGPSVFLFPPKPKDTLMISRTPEVTCVVVDVSHEDPEVKFNWYVDGVEVHNAKTKPREEQYNSTYRVVSVLTVLHQDWLNGKEYKCKVSNKALPAPIEKTISKAKGQPREPQVYTLPPSREEMTKNQVSLTCLVKGFYPSDIAVEWESNGQPENNYKTTPPVLDSDGSFFLYSKLTVDKSRWQQGNVFSCSVMHEALHNHYTQKSLSLSPGGGGGSGGGGSGGGGSGGGGSDIQMTQSPSSLSASVGDRVTITCRASQHVSTAVNWYQQKPGKAPKLLIYSASYLYSGVPSRFSGSRSGTDFTLTISSLQPEDFATYYCQQHYITPYTFGCGTKLEIKGGGGSGGGGSGGGGSQVQLQESGPGLVKPSETLSLTCTVSGYSITSDYAWIWIRQPPGKCLEWIGYITSSGSTYYNPSLKSRVTFSVDTSKNQFSLKLSSVTAADTATYYCARLDFGNYGGAMDYWGQGTLVTVSS

SEQ ID NO: 86 - protein, 717 aa, Artificial Sequence
  900692 heavy chain
QVQLVQSGAEVKKPGASVKVSCKASGYAFTGYTIHWVRQAPGQRLEWMGWFYPGSGTLKYSEKFQGRVTITRDKSLSTAYMELSSLRSEDTAVYYCARHGTGTLMAMDYWGQGTLVTVSSASTKGPSVFPLAPSSKSTSGGTAALGCLVKDYFPEPVTVSWNSGALTSGVHTFPAVLQSSGLYSLSSVVTVPSSSLGTQTYICNVNHKPSNTKVDKRVEPKSCDKTHTCPPCPAPELLGGPSVFLFPPKPKDTLMISRTPEVTCVVVDVSHEDPEVKFNWYVDGVEVHNAKTKPREEQYNSTYRVVSVLTVLHQDWLNGKEYKCKVSNKALPAPIEKTISKAKGQPREPQVYTLPPSREEMTKNQVSLTCLVKGFYPSDIAVEWESNGQPENNYKTTPPVLDSDGSFFLYSKLTVDKSRWQQGNVFSCSVMHEALHNHYTQKSLSLSPGGGGGSGGGGSGGGGSGGGGSDIQMTQSPSSLSASVGDRVTITCRASQHVSTAVNWYQQKPGKAPKLLIYSASYLYSGVPSRFSGSRSGTDFTLTISSLQPEDFATYYCQQHYITPYTFGCGTKLEIKGGGGSGGGGSGGGGSGGGGSQVQLQESGPGLVKPSETLSLTCTVSGYSITSDYAWIWIRQPPGKCLEWIGYITSSGSTYYNPSLKSRVTFSVDTSKNQFSLKLSSVTAADTATYYCARLDFGNYGGAMDYWGQGTLVTVSS

SEQ ID NO: 87 - protein, 722 aa, Artificial Sequence
  900693 heavy chain
QVQLVQSGAEVKKPGASVKVSCKASGYAFTGYTIHWVRQAPGQRLEWMGWFYPGSGTLKYSEKFQGRVTITRDKSLSTAYMELSSLRSEDTAVYYCARHGTGTLMAMDYWGQGTLVTVSSASTKGPSVFPLAPSSKSTSGGTAALGCLVKDYFPEPVTVSWNSGALTSGVHTFPAVLQSSGLYSLSSVVTVPSSSLGTQTYICNVNHKPSNTKVDKRVEPKSCDKTHTCPPCPAPELLGGPSVFLFPPKPKDTLMISRTPEVTCVVVDVSHEDPEVKFNWYVDGVEVHNAKTKPREEQYNSTYRVVSVLTVLHQDWLNGKEYKCKVSNKALPAPIEKTISKAKGQPREPQVYTLPPSREEMTKNQVSLTCLVKGFYPSDIAVEWESNGQPENNYKTTPPVLDSDGSFFLYSKLTVDKSRWQQGNVFSCSVMHEALHNHYTQKSLSLSPGGGGGSGGGGSGGGGSGGGGSDIQMTQSPSSLSASVGDRVTITCRASQHVSTAVNWYQQKPGKAPKLLIYSASYLYSGVPSRFSGSRSGTDFTLTISSLQPEDFATYYCQQHYITPYTFGCGTKLEIKGGGGSGGGGSGGGGSGGGGSGGGGSQVQLQESGPGLVKPSETLSLTCTVSGYSITSDYAWIWIRQPPGKCLEWIGYITSSGSTYYNPSLKSRVTFSVDTSKNQFSLKLSSVTAADTATYYCARLDFGNYGGAMDYWGQGTLVTVSS

SEQ ID NO: 88 - protein, 219 aa, Artificial Sequence
  900339 light chain
DVVMTQTPLSLSVTPGQPASISCKSSQSLANSYGNTYLSWYLHKPGQSPQLLIYGISNRFSGVPDRFSGSGSGTDFTLKISRVEAEDVGVYYCLQGTHQPPTFGQGTKLEIKRTVAAPSVFIFPPSDEQLKSGTASVVCLLNNFYPREAKVQWKVDNALQSGNSQESVTEQDSKDSTYSLSSTLTLSKADYEKHKVYACEVTHQGLSSPVTKSFNRGEC

SEQ ID NO: 89 - protein, 247 aa, Artificial Sequence
  (900339-VL)-Linker1-(900339-VH)
DVVMTQTPLSLSVTPGQPASISCKSSQSLANSYGNTYLSWYLHKPGQSPQLLIYGISNRFSGVPDRFSGSGSGTDFTLKISRVEAEDVGVYYCLQGTHQPPTFGQGTKLEIKGGGGSGGGGSGGGGSQVQLVQSGAEVKKPGASVKVSCKASGYAFTGYTIHWVRQAPGQRLEWMGWFYPGSGTLKYSEKFQGRVTITRDKSLSTAYMELSSLRSEDTAVYYCARHGTGTLMAMDYWGQGTLVTVSS

SEQ ID NO: 90 - protein, 247 aa, Artificial Sequence
  (900339-VL-Q100C)-Linker1-(900339-VH-R44C)
DVVMTQTPLSLSVTPGQPASISCKSSQSLANSYGNTYLSWYLHKPGQSPQLLIYGISNRFSGVPDRFSGSGSGTDFTLKISRVEAEDVGVYYCLQGTHQPPTFGCGTKLEIKGGGGSGGGGSGGGGSQVQLVQSGAEVKKPGASVKVSCKASGYAFTGYTIHWVRQAPGQCLEWMGWFYPGSGTLKYSEKFQGRVTITRDKSLSTAYMELSSLRSEDTAVYYCARHGTGTLMAMDYWGQGTLVTVSS

SEQ ID NO: 91 - protein, 252 aa, Artificial Sequence
  (900339-VL)-Linker2-(900339-VH)
DVVMTQTPLSLSVTPGQPASISCKSSQSLANSYGNTYLSWYLHKPGQSPQLLIYGISNRFSGVPDRFSGSGSGTDFTLKISRVEAEDVGVYYCLQGTHQPPTFGQGTKLEIKGGGGSGGGGSGGGGSGGGGSQVQLVQSGAEVKKPGASVKVSCKASGYAFTGYTIHWVRQAPGQRLEWMGWFYPGSGTLKYSEKFQGRVTITRDKSLSTAYMELSSLRSEDTAVYYCARHGTGTLMAMDYWGQGTLVTVSS

SEQ ID NO: 92 - protein, 252 aa, Artificial Sequence
  (900339-VL-Q100C)-Linker2-(900339-VH-R44C)
DVVMTQTPLSLSVTPGQPASISCKSSQSLANSYGNTYLSWYLHKPGQSPQLLIYGISNRFSGVPDRFSGSGSGTDFTLKISRVEAEDVGVYYCLQGTHQPPTFGCGTKLEIKGGGGSGGGGSGGGGSGGGGSQVQLVQSGAEVKKPGASVKVSCKASGYAFTGYTIHWVRQAPGQCLEWMGWFYPGSGTLKYSEKFQGRVTITRDKSLSTAYMELSSLRSEDTAVYYCARHGTGTLMAMDYWGQGTLVTVSS

SEQ ID NO: 93 - protein, 257 aa, Artificial Sequence
  (900339-VL)-Linker3-(900339-VH)
DVVMTQTPLSLSVTPGQPASISCKSSQSLANSYGNTYLSWYLHKPGQSPQLLIYGISNRFSGVPDRFSGSGSGTDFTLKISRVEAEDVGVYYCLQGTHQPPTFGQGTKLEIKGGGGSGGGGSGGGGSGGGGSGGGGSQVQLVQSGAEVKKPGASVKVSCKASGYAFTGYTIHWVRQAPGQRLEWMGWFYPGSGTLKYSEKFQGRVTITRDKSLSTAYMELSSLRSEDTAVYYCARHGTGTLMAMDYWGQGTLVTVSS

SEQ ID NO: 94 - protein, 257 aa, Artificial Sequence
  (900339-VL-Q100C)-Linker3-(900339-VH-R44C)
DVVMTQTPLSLSVTPGQPASISCKSSQSLANSYGNTYLSWYLHKPGQSPQLLIYGISNRFSGVPDRFSGSGSGTDFTLKISRVEAEDVGVYYCLQGTHQPPTFGCGTKLEIKGGGGSGGGGSGGGGSGGGGSGGGGSQVQLVQSGAEVKKPGASVKVSCKASGYAFTGYTIHWVRQAPGQCLEWMGWFYPGSGTLKYSEKFQGRVTITRDKSLSTAYMELSSLRSEDTAVYYCARHGTGTLMAMDYWGQGTLVTVSS

SEQ ID NO: 95 - protein, 262 aa, Artificial Sequence
  (900339-VL)-Linker4-(900339-VH)
DVVMTQTPLSLSVTPGQPASISCKSSQSLANSYGNTYLSWYLHKPGQSPQLLIYGISNRFSGVPDRFSGSGSGTDFTLKISRVEAEDVGVYYCLQGTHQPPTFGQGTKLEIKGGGGSGGGGSGGGGSGGGGSGGGGSGGGGSQVQLVQSGAEVKKPGASVKVSCKASGYAFTGYTIHWVRQAPGQRLEWMGWFYPGSGTLKYSEKFQGRVTITRDKSLSTAYMELSSLRSEDTAVYYCARHGTGTLMAMDYWGQGTLVTVSS

SEQ ID NO: 96 - protein, 262 aa, Artificial Sequence
  (900339-VL-Q100C)-Linker4-(900339-VH-R44C)
DVVMTQTPLSLSVTPGQPASISCKSSQSLANSYGNTYLSWYLHKPGQSPQLLIYGISNRFSGVPDRFSGSGSGTDFTLKISRVEAEDVGVYYCLQGTHQPPTFGCGTKLEIKGGGGSGGGGSGGGGSGGGGSGGGGSGGGGSQVQLVQSGAEVKKPGASVKVSCKASGYAFTGYTIHWVRQAPGQCLEWMGWFYPGSGTLKYSEKFQGRVTITRDKSLSTAYMELSSLRSEDTAVYYCARHGTGTLMAMDYWGQGTLVTVSS

SEQ ID NO: 97 - protein, 243 aa, Artificial Sequence
  (HB0030-VL-Q100C)-Linker1-(HB0030-VH-G44C)
DIQMTQSPSSLSASVGDRVTITCRASQHVSTAVNWYQQKPGKAPKLLIYSASYLYSGVPSRFSGSRSGTDFTLTISSLQPEDFATYYCQQHYITPYTFGCGTKLEIKGGGGSGGGGSGGGGSQVQLQESGPGLVKPSETLSLTCTVSGYSITSDYAWIWIRQPPGKCLEWIGYITSSGSTYYNPSLKSRVTFSVDTSKNQFSLKLSSVTAADTATYYCARLDFGNYGGAMDYWGQGTLVTVSS

SEQ ID NO: 98 - protein, 248 aa, Artificial Sequence
  (HB0030-VL-Q100C)-Linker2-(HB0030-VH-G44C)
DIQMTQSPSSLSASVGDRVTITCRASQHVSTAVNWYQQKPGKAPKLLIYSASYLYSGVPSRFSGSRSGTDFTLTISSLQPEDFATYYCQQHYITPYTFGCGTKLEIKGGGGSGGGGSGGGGSGGGGSQVQLQESGPGLVKPSETLSLTCTVSGYSITSDYAWIWIRQPPGKCLEWIGYITSSGSTYYNPSLKSRVTFSVDTSKNQFSLKLSSVTAADTATYYCARLDFGNYGGAMDYWGQGTLVTVSS

SEQ ID NO: 99 - protein, 253 aa, Artificial Sequence
  (HB0030-VL-Q100C)-Linker3-(HB0030-VH-G44C)
DIQMTQSPSSLSASVGDRVTITCRASQHVSTAVNWYQQKPGKAPKLLIYSASYLYSGVPSRFSGSRSGTDFTLTISSLQPEDFATYYCQQHYITPYTFGCGTKLEIKGGGGSGGGGSGGGGSGGGGSGGGGSQVQLQESGPGLVKPSETLSLTCTVSGYSITSDYAWIWIRQPPGKCLEWIGYITSSGSTYYNPSLKSRVTFSVDTSKNQFSLKLSSVTAADTATYYCARLDFGNYGGAMDYWGQGTLVTVSS

SEQ ID NO: 100 - protein, 8 aa, Artificial Sequence
  PD-L1 HCDR1
GYAFTGYT

SEQ ID NO: 101 - protein, 8 aa, Artificial Sequence
  PD-L1 HCDR2
FYPGSGTL

SEQ ID NO: 102 - protein, 13 aa, Artificial Sequence
  PD-L1 HCDR3
ARHGTGTLMAMDY

SEQ ID NO: 103 - protein, 11 aa, Artificial Sequence
  PD-L1 LCDR1
QSLANSYGNTY

SEQ ID NO: 104 - protein, 3 aa, Artificial Sequence
  PD-L1 LCDR2
GIS

SEQ ID NO: 105 - protein, 9 aa, Artificial Sequence
  PD-L1 LCDR3
LQGTHQPPT

SEQ ID NO: 106 - protein, 120 aa, Artificial Sequence
  PD-L1 VH
QVQLVQSGAEVKKPGASVKVSCKASGYAFTGYTIHWVRQAPGQRLEWMGWFYPGSGTLKYSEKFQGRVTITRDKSLSTAYMELSSLRSEDTAVYYCARHGTGTLMAMDYWGQGTLVTVSS

SEQ ID NO: 107 - protein, 112 aa, Artificial Sequence
  PD-L1 VL
DVVMTQTPLSLSVTPGQPASISCKSSQSLANSYGNTYLSWYLHKPGQSPQLLIYGISNRFSGVPDRFSGSGSGTDFTLKISRVEAEDVGVYYCLQGTHQPPTFGQGTKLEIK

SEQ ID NO: 108 - protein, 120 aa, Artificial Sequence
  PD-L1 VH R44C
QVQLVQSGAEVKKPGASVKVSCKASGYAFTGYTIHWVRQAPGQCLEWMGWFYPGSGTLKYSEKFQGRVTITRDKSLSTAYMELSSLRSEDTAVYYCARHGTGTLMAMDYWGQGTLVTVSS

SEQ ID NO: 109 - protein, 112 aa, Artificial Sequence
  PD-L1 VL Q100C
DVVMTQTPLSLSVTPGQPASISCKSSQSLANSYGNTYLSWYLHKPGQSPQLLIYGISNRFSGVPDRFSGSGSGTDFTLKISRVEAEDVGVYYCLQGTHQPPTFGCGTKLEIK

SEQ ID NO: 110 - protein, 121 aa, Artificial Sequence
  HB0030 VH G44C
QVQLQESGPGLVKPSETLSLTCTVSGYSITSDYAWIWIRQPPGKCLEWIGYITSSGSTYYNPSLKSRVTFSVDTSKNQFSLKLSSVTAADTATYYCARLDFGNYGGAMDYWGQGTLVTVSS

SEQ ID NO: 111 - protein, 107 aa, Artificial Sequence
  HB0030 VL Q100C
DIQMTQSPSSLSASVGDRVTITCRASQHVSTAVNWYQQKPGKAPKLLIYSASYLYSGVPSRFSGSRSGTDFTLTISSLQPEDFATYYCQQHYITPYTFGCGTKLEIK